European Patent Application EP 4 751 739 A1, published June 3, 2026. Title: 靶向c-Met的抗体-药物偶联物及其医药用途. Applicant: 江苏恒瑞医药股份有限公司. Application WO. The sequence listing filed with the application follows.

SEQUENCE LISTING (22 sequences)

SEQ ID NO: 1 - protein, 5 aa, synthetic construct
  source 1..5: note = HCDR1
NYGVH

SEQ ID NO: 2 - protein, 16 aa, synthetic construct
  source 1..16: note = HCDR2
VIWSGGSTNYAAAFVS

SEQ ID NO: 3 - protein, 12 aa, synthetic construct
  source 1..12: note = HCDR3
NHDNPYNYAMDY

SEQ ID NO: 4 - protein, 15 aa, synthetic construct
  source 1..15: note = LCDR1
RANKSVSTSTYNYLH

SEQ ID NO: 5 - protein, 7 aa, synthetic construct
  source 1..7: note = LCDR2
LASNLAS

SEQ ID NO: 6 - protein, 9 aa, synthetic construct
  source 1..9: note = LCDR3
QHSRDLPPT

SEQ ID NO: 7 - protein, 15 aa, synthetic construct
  source 1..15: note = LCDR1
RADKSVSTSTYNYLH

SEQ ID NO: 8 - protein, 120 aa, synthetic construct
  source 1..120: note = VH
QVQLKQSGPGLVQPSQSLSITCTVSGFSLPNYGVHWVRQSPGKGLEWLGVIWSGGSTNYAAAFVSRLRISKDNSKSQVFFEMNSLQADDTAVYYCARNHDNPYNYAMDYWGQGTTVTVSS

SEQ ID NO: 9 - protein, 112 aa, synthetic construct
  source 1..112: note = VL
DIVLTQSPGSLAVYLGQRATISCRANKSVSTSTYNYLHWYQQKPGQPPKLLIYLASNLASGVPARFSGSGSGTDFTLNIHPLEEEDAATYYCQHSRDLPPTFGAGTKLELKR

SEQ ID NO: 10 - protein, 120 aa, synthetic construct
  source 1..120: note = Ab-9 VH
QVTLKESGPVLVKPTETLTLTCTVSGFSLPNYGVHWVRQPPGKALEWLAVIWSGGSTNYAAAFVSRLRISKDTSKSQVVFTMNNMDPVDTATYYCARNHDNPYNYAMDYWGQGTTVTVSS

SEQ ID NO: 11 - protein, 120 aa, synthetic construct
  source 1..120: note = Ab-10 VH
QVQLVESGGGVVQPGRSLRLSCAASGFSLSNYGVHWVRQAPGKGLEWLAVIWSGGSTNYAAAFVSRLTISKDNSKNTVYLQMNSLRAEDTAVYYCARNHDNPYNYAMDYWGQGTTVTVSS

SEQ ID NO: 12 - protein, 120 aa, synthetic construct
  source 1..120: note = Ab-11 VH
QVQLVESGGGVVQPGRSLRLSCAASGFTLPNYGVHWVRQAPGKGLEWLAVIWSGGSTNYAAAFVSRLTISKDNSKNTVYLQMNSLRAEDTAVYYCARNHDNPYNYAMDYWGQGTTVTVSS

SEQ ID NO: 13 - protein, 112 aa, synthetic construct
  source 1..112: note = Ab-9 VL
DIVLTQSPASLAVSPGQRATITCRANKSVSTSTYNYLHWYQQKPGQPPKLLIYLASNLASGVPARFSGSGSGTDFTLTINPVEANDTANYYCQHSRDLPPTFGQGTKLEIKR

SEQ ID NO: 14 - protein, 112 aa, synthetic construct
  source 1..112: note = Ab-10 VL
DIVLTQSPDSLAVSLGERATINCRADKSVSTSTYNYLHWYQQKPGQPPKLLIYLASNLASGVPDRFSGSGSGTDFTLTISSLQAEDVAVYYCQHSRDLPPTFGQGTKLEIKR

SEQ ID NO: 15 - protein, 112 aa, synthetic construct
  source 1..112: note = Ab-11 VL
DIVLTQSPDSLAVSLGERATINCRANKSVSTSTYNYLHWYQQKPGQPPKLLIYLASNLASGVPDRFSGSGSGTDFTLTISSLQAEDVAVYYCQHSRDLPPTFGQGTKLEIKR

SEQ ID NO: 16 - protein, 446 aa, synthetic construct
  source 1..446: note = Ab-9 HC
QVTLKESGPVLVKPTETLTLTCTVSGFSLPNYGVHWVRQPPGKALEWLAVIWSGGSTNYAAAFVSRLRISKDTSKSQVVFTMNNMDPVDTATYYCARNHDNPYNYAMDYWGQGTTVTVSSASTKGPSVFPLAPCSRSTSESTAALGCLVKDYFPEPVTVSWNSGALTSGVHTFPAVLQSSGLYSLSSVVTVPSSNFGTQTYTCNVDHKPSNTKVDKTVERKCCVECPPCPAPPVAGPSVFLFPPKPKDTLMISRTPEVTCVVVDVSHEDPEVQFNWYVDGVEVHNAKTKPREEQFNSTFRVVSVLTVVHQDWLNGKEYKCKVSNKGLPAPIEKTISKTKGQPREPQVYTLPPSREEMTKNQVSLTCLVKGFYPSDIAVEWESNGQPENNYKTTPPMLDSDGSFFLYSKLTVDKSRWQQGNVFSCSVMHEALHNHYTQKSLSLSPGK

SEQ ID NO: 17 - protein, 218 aa, synthetic construct
  source 1..218: note = Ab-9 LC
DIVLTQSPASLAVSPGQRATITCRANKSVSTSTYNYLHWYQQKPGQPPKLLIYLASNLASGVPARFSGSGSGTDFTLTINPVEANDTANYYCQHSRDLPPTFGQGTKLEIKRTVAAPSVFIFPPSDEQLKSGTASVVCLLNNFYPREAKVQWKVDNALQSGNSQESVTEQDSKDSTYSLSSTLTLSKADYEKHKVYACEVTHQGLSSPVTKSFNRGEC

SEQ ID NO: 18 - protein, 446 aa, synthetic construct
  source 1..446: note = Ab-10 HC
QVQLVESGGGVVQPGRSLRLSCAASGFSLSNYGVHWVRQAPGKGLEWLAVIWSGGSTNYAAAFVSRLTISKDNSKNTVYLQMNSLRAEDTAVYYCARNHDNPYNYAMDYWGQGTTVTVSSASTKGPSVFPLAPCSRSTSESTAALGCLVKDYFPEPVTVSWNSGALTSGVHTFPAVLQSSGLYSLSSVVTVPSSNFGTQTYTCNVDHKPSNTKVDKTVERKCCVECPPCPAPPVAGPSVFLFPPKPKDTLMISRTPEVTCVVVDVSHEDPEVQFNWYVDGVEVHNAKTKPREEQFNSTFRVVSVLTVVHQDWLNGKEYKCKVSNKGLPAPIEKTISKTKGQPREPQVYTLPPSREEMTKNQVSLTCLVKGFYPSDIAVEWESNGQPENNYKTTPPMLDSDGSFFLYSKLTVDKSRWQQGNVFSCSVMHEALHNHYTQKSLSLSPGK

SEQ ID NO: 19 - protein, 218 aa, synthetic construct
  source 1..218: note = Ab-10 LC
DIVLTQSPDSLAVSLGERATINCRADKSVSTSTYNYLHWYQQKPGQPPKLLIYLASNLASGVPDRFSGSGSGTDFTLTISSLQAEDVAVYYCQHSRDLPPTFGQGTKLEIKRTVAAPSVFIFPPSDEQLKSGTASVVCLLNNFYPREAKVQWKVDNALQSGNSQESVTEQDSKDSTYSLSSTLTLSKADYEKHKVYACEVTHQGLSSPVTKSFNRGEC

SEQ ID NO: 20 - protein, 446 aa, synthetic construct
  source 1..446: note = Ab-11 HC
QVQLVESGGGVVQPGRSLRLSCAASGFTLPNYGVHWVRQAPGKGLEWLAVIWSGGSTNYAAAFVSRLTISKDNSKNTVYLQMNSLRAEDTAVYYCARNHDNPYNYAMDYWGQGTTVTVSSASTKGPSVFPLAPCSRSTSESTAALGCLVKDYFPEPVTVSWNSGALTSGVHTFPAVLQSSGLYSLSSVVTVPSSNFGTQTYTCNVDHKPSNTKVDKTVERKCCVECPPCPAPPVAGPSVFLFPPKPKDTLMISRTPEVTCVVVDVSHEDPEVQFNWYVDGVEVHNAKTKPREEQFNSTFRVVSVLTVVHQDWLNGKEYKCKVSNKGLPAPIEKTISKTKGQPREPQVYTLPPSREEMTKNQVSLTCLVKGFYPSDIAVEWESNGQPENNYKTTPPMLDSDGSFFLYSKLTVDKSRWQQGNVFSCSVMHEALHNHYTQKSLSLSPGK

SEQ ID NO: 21 - protein, 218 aa, synthetic construct
  source 1..218: note = Ab-11 LC
DIVLTQSPDSLAVSLGERATINCRANKSVSTSTYNYLHWYQQKPGQPPKLLIYLASNLASGVPDRFSGSGSGTDFTLTISSLQAEDVAVYYCQHSRDLPPTFGQGTKLEIKRTVAAPSVFIFPPSDEQLKSGTASVVCLLNNFYPREAKVQWKVDNALQSGNSQESVTEQDSKDSTYSLSSTLTLSKADYEKHKVYACEVTHQGLSSPVTKSFNRGEC

SEQ ID NO: 22 - protein, 15 aa, synthetic construct
  source 1..15: note = LCDR1
  VARIANT 3: note = X1=N or D
RAXKSVSTSTYNYLH